European Patent Application EP 4 202 050 A1, published June 28, 2023. Title: Method for the biotechnological production of erythritol. Applicant: Conzil Estate GmbH. The sequence listing filed with the application follows.

SEQUENCE LISTING (22 sequences)

SEQ ID NO: 1 - DNA, 2010 bp, Saccharomyces cerevisiae
atgagcaatccccaaaaggcactgaacgacttcctcagctccgagagcgtccacacccacgactcctcacgtaagcagtccaacaagcaatcctcggacgagggccgtagctcgagccagccctcccaccatcactccggaggaactaataacaataacaacaataacaacaacaacaacaacagcaacaacaacaacaacggtaacgatggcggcaacgacgacgactatgactacgagatgcaggactaccgtccctccccacagtctgctaggcctactcccacctacgtgccccaatacagtgtcgagtcgggcaccgcattccccattcaagaggtcattccctcggcctacattaacacccaagacatcaaccacaaggacaacggccccccttccgcatcgtcaaaccgcgctttccgcccccgcggccagacgaccgtcagcgccaacgtcctgaacatagaggacttctacaagaatgcggacgatgcacacacaattccagagtcgcatctgagccggcgtcgctcccgatcacgggccacgtcaaatgcaggccactccgccaacaccggcgccaccaatggtcgtactacgggcgcccagaccaacatggagagcaacgagtcccccaggaacgtgccgataatggtcaagcctaagaccctctaccagaacccgcagacccccacagttctcccctcaacttaccacccgattaacaagtggagctccgttaagaatacctatttaaaagagttcctcgccgagtttatgggtacgatggtcatgatcatcttcggcagcgccgtcgtatgccaggtcaacgtcgccggcaagatccagcaggacaacttcaacgtagccctcgacaacctcaatgtcacgggctcttccgccgagacaatcgacgccatgaagagcctgactagcctagtctcctctgtcgccggtggcaccttcgatgacgttgccctcgggtgggccgctgccgtggtaatgggctacttttgtgcaggtggctcggcaatctctggagcccacctgaacccatcaatcaccctcgctaacctcgtttatcgaggctttcccctgaagaaggtcccatattacttcgcaggccagctgattggtgctttcacgggagccctcattctgttcatttggtacaagagggtccttcaggaggcatactcggactggtggatgaacgaatccgtcgctggcatgttttgtgtcttcccaaagccctacctgagctctgggcggcagttttttagcgagttcctctgcggcgccatgctccaggccgggacattcgccctgacggatccctacacgtgcttgagctcagatgtatttcccctgatgatgttcattctcattttcatcattaacgcttcgatggcatatcagacaggtactgcgatgaacctggcacgggatctgggcccccgcctcgccctctacgcagtgggcttcgaccacaagatgctctgggtccaccaccaccacttcttttgggtgccgatggtagggccgtttattggtgccctgatggggggcctcgtctacgacgtctgtatctaccaaggccacgaatcaccggttaactggtctctccccgtgtacaaggaaatgattatgcgcgcatggtttaggcgccccggatggaagaagcggaaccgagctaggaggacttctgacctctccgacttctcttacaataatgacgacgacgaggaattcggcgaacgcatggcgcttcagaagacgaagacgaagtctagcatttccgacaacgagaacgaggccggcgagaagaaggttcagttcaagtccgttcagcgagggaagcggaccttcggcggcatcccgacaattcttgaggaggaggatagcatcgagactgccagcctcggcgccacgacaacggattctattggtctctctgacactagctctgaggacagccactacggcaacgcgaagaaagtcacctga

SEQ ID NO: 2 - protein, 669 aa, Saccharomyces cerevisiae
MSNPQKALNDFLSSESVHTHDSSRKQSNKQSSDEGRSSSQPSHHHSGGTNNNNNNNNNNNNSNNNNNGNDGGNDDDYDYEMQDYRPSPQSARPTPTYVPQYSVESGTAFPIQEVIPSAYINTQDINHKDNGPPSASSNRAFRPRGQTTVSANVLNIEDFYKNADDAHTIPESHLSRRRSRSRATSNAGHSANTGATNGRTTGAQTNMESNESPRNVPIMVKPKTLYQNPQTPTVLPSTYHPINKWSSVKNTYLKEFLAEFMGTMVMIIFGSAVVCQVNVAGKIQQDNFNVALDNLNVTGSSAETIDAMKSLTSLVSSVAGGTFDDVALGWAAAVVMGYFCAGGSAISGAHLNPSITLANLVYRGFPLKKVPYYFAGQLIGAFTGALILFIWYKRVLQEAYSDWWMNESVAGMFCVFPKPYLSSGRQFFSEFLCGAMLQAGTFALTDPYTCLSSDVFPLMMFILIFIINASMAYQTGTAMNLARDLGPRLALYAVGFDHKMLWVHHHHFFWVPMVGPFIGALMGGLVYDVCIYQGHESPVNWSLPVYKEMIMRAWFRRPGWKKRNRARRTSDLSDFSYNNDDDEEFGERMALQKTKTKSSISDNENEAGEKKVQFKSVQRGKRTFGGIPTILEEEDSIETASLGATTTDSIGLSDTSSEDSHYGNAKKVT

SEQ ID NO: 3 - DNA, 996 bp, Trichoderma reesei
atgtcttccggaaggaccgtcaccctcaacaccggctacaagatcccccagatcggctacggcacctggcaggccgctcccggcgaggtcggcgctggtgtctttgaggccctcaaggttggctaccgccacctcgacctggccaaggtctacggcaaccagaaggaggttggtgagggcatcaagaaggctcttgctgaggtccccggcctgaagcgcgaggatattttcatcacctccaagctgtggaacaactcccacaagcccgaggacgtcgagcccgctctcgacgacaccctggccgagcttggcctcgactaccttgacctctacctcatccactggcccgttgcctttgctcccggcgccgacctcttccccaagtccgaggacggctccgaggtgcagctcaaccagaatgtgtccattgtccagacctggaaggccatgaccgagctgcccaagtccaaggtccgctccgtcggtgtctccaactttaccatagagcacctcgacgccgtcatcgaggccaccggcgtcgtccccgccgtcaaccagatcgagcgccacccccgcctccccaaccagcctctgatcgactactgcgccaagaagggcatcatcatcaccgcctactccgcctttggcaacaacacaaagggcctgcccctgctcgtcagctccgacgaggtcaaggccgtcgccgacaacctgtccaagaagcagggcaagaccgtcactcccgcccaggtcatcctcgcctggtcccagattggtggccacaccgtcattcccaagtccgtcaccaaggcgcgcattgcggagaacttccaggaggttgagctggatgacgaggccattgctgcgctgaacaagttgggcgagaagcctcagcggttcaacattccttacacctacaagcctaggtggaacattaacctgttcaacaccgaggaggagaaggccgctgcccacactgctgtcatcaagctgtaa

SEQ ID NO: 4 - protein, 331 aa, Trichoderma reesei
MSSGRTVTLNTGYKIPQIGYGTWQAAPGEVGAGVFEALKVGYRHLDLAKVYGNQKEVGEGIKKALAEVPGLKREDIFITSKLWNNSHKPEDVEPALDDTLAELGLDYLDLYLIHWPVAFAPGADLFPKSEDGSEVQLNQNVSIVQTWKAMTELPKSKVRSVGVSNFTIEHLDAVIEATGVVPAVNQIERHPRLPNQPLIDYCAKKGIIITAYSAFGNNTKGLPLLVSSDEVKAVADNLSKKQGKTVTPAQVILAWSQIGGHTVIPKSVTKARIAENFQEVELDDEAIAALNKLGEKPQRFNIPYTYKPRWNINLFNTEEEKAAAHTAVIKL

SEQ ID NO: 5 - DNA, 2055 bp, Trichoderma reesei
atgggctacacagaggttgaccagaaggccatcaacaccatccgcctgctcgcggtcgatgccaccttcaagagcaactcgggccacccgggtgcccccatgggcatggctcccgttgcccacgtcctttgggacaagttcatgaggttcaaccccaagaaccccaagtggctgaaccgtgaccgattcgttctctccaacggccacggctgcatgctccagtatgctctgcttcacctgttcggctacgacctgaccatcgatgacctcaaggccttccgaaccgtcgacagcaagactcctggtcaccccgaggcccacgatactcccggtgtcgaggtcaccaccggccccctgggtcagggtatctccaatgccgtcggtctggccatggcccaggcccacaccgccgccaccttcaacaagcccggcttcaccctgtgtgacaactacacctactgcttcctcggcgatggctgcttgatggagggtgtctctgccgaggcctcgtccctggccggccacctccagctcggcaacctcatctgcatctacgatgacaaccacatctccattgacggcgacaccaactgtgccttcaccgaggacgtggccaagcgctacgaggcctacggctggcacgtcgaggtcgtcgagaacggcgaccacgacctcgaggccatggaggccgccatcaagaagtgccaggaggtcaaggacaagccctcaatcatcaagctgcgcaccaccattggcttcggctctctccaggagggcacccacggagtccacggctctcccctcaaggccgacgacatcaagcagctcaagcagaagtttggcttcaaccccgacgagagcttcgtcgtccccaaggaggtctccgacctctacgcccgccactcagccgagggcgccgccgccgaggaggagtggaacaagctgttcgccaagtacgccgagaagtaccccgccgaggctgctgacctccagcgccgcctcaagggcgagctgcccgagggctgggagaagaacctgcccgtctactcgcccagcgatgctgccattgccagccgaaagctgtccgagacggtcctcaccaagatccacgacgtcctgcccgagctccagggtggttccgccgatctgactggttccaacctgacccgctggaaggacgctgttgacttccagccccccgccaccggcctcggtgactactccggacgatacatccgctacggtgtccgcgagcacggcatgggcgccatcatgaacggcctggccgcctacggcaccatcatcccctacggcggtaccttcctcaacttcgtctcctacgccgccggtgccgtccgcctgtccgctctgtcccgcgtccgcgtcatctgggtcgccacccacgactccattggcctgggcgaggacggtcctactcaccagcctatcgagactctggctcacttccgcgccctgcccaactgcatggtgtggcgccccgccgacggcaacgagaccagcgctgcctactacattgccctgacctccaagcacacccccagcatcattgccctgtctcgccagaacctgccccagctcgagggctccgtcatcgagaaggccatcaagggaggatacgtcctgcaggaggtcgagggtgcccagatcaccctggtctccaccggttccgaggtttccatcgccgtggatgccgccaagtacctcctggagaagcacaacgtcaaggcccgcgtcgtctccatgccctgcttcgaggttttcgatgctcagcccaaggagtacagactctccgtcctgcccgacggcatcccctctctgtccattgaggtgatgagcaccatgggctgggagcgatacactcacgagcagtttggtctcaaccgattcggtgcctctggcgcctacaaggatgtctacaagaagttcgagttcacccccgagggcatcaccaagcgcgctcttctcaccattgacttctggaaggacgtccccaacgtccgctctcccatcaaccgtgccttccagcagctcatc

SEQ ID NO: 6 - protein, 685 aa, Trichoderma reesei
MGYTEVDQKAINTIRLLAVDATFKSNSGHPGAPMGMAPVAHVLWDKFMRFNPKNPKWLNRDRFVLSNGHGCMLQYALLHLFGYDLTIDDLKAFRTVDSKTPGHPEAHDTPGVEVTTGPLGQGISNAVGLAMAQAHTAATFNKPGFTLCDNYTYCFLGDGCLMEGVSAEASSLAGHLQLGNLICIYDDNHISIDGDTNCAFTEDVAKRYEAYGWHVEVVENGDHDLEAMEAAIKKCQEVKDKPSIIKLRTTIGFGSLQEGTHGVHGSPLKADDIKQLKQKFGFNPDESFVVPKEVSDLYARHSAEGAAAEEEWNKLFAKYAEKYPAEAADLQRRLKGELPEGWEKNLPVYSPSDAAIASRKLSETVLTKIHDVLPELQGGSADLTGSNLTRWKDAVDFQPPATGLGDYSGRYIRYGVREHGMGAIMNGLAAYGTIIPYGGTFLNFVSYAAGAVRLSALSRVRVIWVATHDSIGLGEDGPTHQPIETLAHFRALPNCMVWRPADGNETSAAYYIALTSKHTPSIIALSRQNLPQLEGSVIEKAIKGGYVLQEVEGAQITLVSTGSEVSIAVDAAKYLLEKHNVKARVVSMPCFEVFDAQPKEYRLSVLPDGIPSLSIEVMSTMGWERYTHEQFGLNRFGASGAYKDVYKKFEFTPEGITKRALLTIDFWKDVPNVRSPINRAFQQLI

SEQ ID NO: 7 - DNA, 975 bp, Trichoderma reesei
atgagctcctctcttgaccagctcaaggccactggcaccgttgtcgtctctgacactggtgactttgctgccatcgccaagtacaagccccaggatgccaccaccaacccctccctcatcctggccgcctccaagaagcccgagtacgccaagctgatagacgtcgccatcgactacgccaagcagaagggcggcgacattgagcagcaggtcgacgatgccctcgaccgcctgctggtcgagttcggcaaggagattctcaagattgttcccggcaaggtctccaccgaggtcgacgcccggttctcctttgacaccaaggcctctgtcgacaaggccctccacattatcgagctctacaaggagctcggcatccccaaggagcgcgtcctcatcaagatcgcctccacctgggagggcatcaaggccgccgagatcctgcagcgcgaccacggcatcaactgcaacctgacgctcatgttctccctgccccaggccatcggcgccgccgaggccggcgccttcctcatctcccccttcgttggccgcatcctcgactggttcaaggcgagcaccaagaaggactactccaaggaggaggaccccggtgtcgcctccgtcaagagcatcttcaactactacaagaagtttggctacaagaccattgtcatgggtgcctcgttccgcaacacgggcgagattaccgagctcgctggctgcgactacctgaccatttctcccaacctgctcgaggagctcctcaactccaccgagcccgtccccaagaagctcgacgccgccgccgctgcctcccttaacattgagaagaagtcgtacatcaacgacgagtccctgttccgcttcgacttcaacgaggaccagatggccgtcgagaagctgcgcgagggcatcagcaagtttgccgccgacgccgtcaccctcaaggacattctgaggcagaagctgtctgcttaa

SEQ ID NO: 8 - protein, 324 aa, Trichoderma reesei
MSSSLDQLKATGTVVVSDTGDFAAIAKYKPQDATTNPSLILAASKKPEYAKLIDVAIDYAKQKGGDIEQQVDDALDRLLVEFGKEILKIVPGKVSTEVDARFSFDTKASVDKALHIIELYKELGIPKERVLIKIASTWEGIKAAEILQRDHGINCNLTLMFSLPQAIGAAEAGAFLISPFVGRILDWFKASTKKDYSKEEDPGVASVKSIFNYYKKFGYKTIVMGASFRNTGEITELAGCDYLTISPNLLEELLNSTEPVPKKLDAAAAASLNIEKKSYINDESLFRFDFNEDQMAVEKLREGISKFAADAVTLKDILRQKLSA

SEQ ID NO: 9 - DNA, 1615 bp, Trichoderma reesei
ctacaaccaccacatcgccaactcttccttctgcaactccaactccttcacttctcttctctgttctactcttctccacctacttcacctaccgcaatcatggccaacgcaactggcaagaaggcagtccactttggcgccggcaacatcggccgtggcttcgttgcttgcttcctccacaactcgggctatgaggtcgtttttgccgacgtcaacggagacctgattgataccatcaactctaccccctcctacaaagtcatcgaggtcggctccgagggcacctcagaaaacgtcatcaccaactaccgggccatcaactctcggactcacgaggaagacctcgttgaggagatccgcactgccgacgtcgtcacctgctccgtcggccccaacatcctcaagttcatcgctcccgtcatcgcaaagggcatcgaccgccgctccgacgacgagacgcccctgcacgtcattgcctgcgagaacgccattggcgccaccgacacgctggccagctacatcaaggatgccaagaacacggatcctgcccgtctcgagacgcaccacctgcgtgcccgctacgccaactcggctattgaccggatcgtgccggcgcaggaccccaatgccggccttgacgtgaagctggagaagttctttgagtgggttgtcgacaagaccccctttgaggacattggcatcccgcccattgagggcatccagtgggtcgacaacctggagcccttcatcgagcgcaagctgtacacggtcaacactggccacgctacggctgcctaccacggctactaccgcagaaagcgcaccgtctacgatgctctccaggacaaggagatcatggctgaggtccgtggcgccctgaccgagaccaagaacctgctcgttgccaagcacggcatcgacgaggaggcccagctcgcctacatgaacaagattatcaagcgcatcggcaacccccatttggaggatgctgtcgagcgtgtcggccgcgctcccctgaggaagctgtcgcgcaaggagcgcttcatcggccccgccgccgaggccgccgagaacgacatgcccgtcaagtacctcctcgacgccatcgagatgacgttccgcttccaggacgtcgagggtgacgacgagtccaaggagctctctaccatcatgtccgagaacacccccgaggacgttgtcgccaaggtctgcggcatcaagccgacggagaagatctaccctcgcctggtcgaggttgtcaagcgtgtgcaggctgacagccaggaggagtaacttgcgatggctcttctggcgttctagctcggcatcactcacggcgctgagtggtgaccggcctactgcatctggctttgggcttcttttgatcttttacttctactttttctcttctacaacttgtgttaagaatgcacgaatgaacggcaaggcgctgggttccgggttaatagagcatcgtctcttttgttttctattttttttgtactctgctagggcattccttgacgggaacaaaaggtgctcgggatatcttcatgggaagcttcagtctatagatggactgagcaggcagcataacgggtcaagataccacatc

SEQ ID NO: 10 - protein, 397 aa, Trichoderma reesei
MANATGKKAVHFGAGNIGRGFVACFLHNSGYEVVFADVNGDLIDTINSTPSYKVIEVGSEGTSENVITNYRAINSRTHEEDLVEEIRTADVVTCSVGPNILKFIAPVIAKGIDRRSDDETPLHVIACENAIGATDTLASYIKDAKNTDPARLETHHLRARYANSAIDRIVPAQDPNAGLDVKLEKFFEWVVDKTPFEDIGIPPIEGIQWVDNLEPFIERKLYTVNTGHATAAYHGYYRRKRTVYDALQDKEIMAEVRGALTETKNLLVAKHGIDEEAQLAYMNKIIKRIGNPHLEDAVERVGRAPLRKLSRKERFIGPAAEAAENDMPVKYLLDAIEMTFRFQDVEGDDESKELSTIMSENTPEDVVAKVCGIKPTEKIYPRLVEVVKRVQADSQEE

SEQ ID NO: 11 - DNA, 1418 bp, Trichoderma reesei
cagacaactacaaacaagatggttggcgttgacgcagagattatcgccgatgataccagaatcctgggtcaggatcctttgatccccccggctctgctcatctccgagatccccatgactcccaatgccctccagaccgtcgtcaagggccggagagacgctgcccagatcatcatgggccagaacgacaggctattagtcgtcgtcggtccctgctccatccacgaccccgaagccgcccacgagtacgccgcccgcctcaagcagctctccgagaagctcgccgacgacctctgcatcgtgatgcgcgcctacctggagaagcctcgcacgaccgtcggctggaagggcctgatcaacgatcccgatatcgactcgtccttccagatcaacaagggcctgcgcgtctcccgccggctcttcgtcgacctgacctccaacggcatgcccattgccaccgagatgctcgacaccatctccccccagttcctcgccgactgcatctccgtcggcgccattggcgcgcgaacgaccgagtcccagctgcaccgtgagctcgcttccggcctgtccttccccgtgggcttcaagaacggaaccgacggcagccttggcgtcgccattgatgccattggcgctgccgcggccaagcaccacttcatgggtgtgacgaagcagggcctggctgccattacccgcaccaagggcaacgagcacggcttcgtgatcctgagaggcggaagcaagggccccaactttgacaaggagagcgtccaggcggccaagaagatgctgacggacaagggccagaagctggccattatgattgactgttctcacggcaactctcagaagaaccacaacaaccagcccaaggttgccaaggccattgccgaccagctgcgcgagggcgagcgagccattgtcggcgtcatgatcgagtccaacatcaacgagggcaaccaaaaggtccctgctgagggtccggccggtctcaagcgcggcgttagcatcacggatgcatgcatcaactgggaggacacagtcacggtcctcgaggaccttgccgctgccgtccgcacccgacgcgaggtcaactcgggtgctcctagcgcagaggccaaggtgagcactctggaggaggactagacgtagttttaccggaaggggcgtatgtgtgtacgatgagagagaggaacgaaaagcatgagggtcggtttgttgattttgaacattacgatgcgtgagtttatgcgcgcgaatcctggcttcctccctggccagcgtaaataagaaaagttttagggagagcattcgacacggatatcgagaaattggcgcaccaaaggaacatgtatgaaggcatatattgttggctgtccactttgtcacagacggcgcacacgaaccagtttcag

SEQ ID NO: 12 - protein, 376 aa, Trichoderma reesei
MVGVDAEIIADDTRILGQDPLIPPALLISEIPMTPNALQTVVKGRRDAAQIIMGQNDRLLVVVGPCSIHDPEAAHEYAARLKQLSEKLADDLCIVMRAYLEKPRTTVGWKGLINDPDIDSSFQINKGLRVSRRLFVDLTSNGMPIATEMLDTISPQFLADCISVGAIGARTTESQLHRELASGLSFPVGFKNGTDGSLGVAIDAIGAAAAKHHFMGVTKQGLAAITRTKGNEHGFVILRGGSKGPNFDKESVQAAKKMLTDKGQKLAIMIDCSHGNSQKNHNNQPKVAKAIADQLREGERAIVGVMIESNINEGNQKVPAEGPAGLKRGVSITDACINWEDTVTVLEDLAAAVRTRREVNSGAPSAEAKVSTLEED

SEQ ID NO: 13 - DNA, 3267 bp, Trichoderma reesei
atgacaacgctgctcaacaacccgccggattcgggtcccccgccgcgccagattcgcttcgtacataaccagggccagccgccgtccaagcgacgcaggatcaatgcagcgtatgttcttctggggcttctctcgccttgcttcgtctgtcttgccgcgtcacccttggtggcaaatggctgtcctagacagataagtgcaagatggcgcgagcatcaacaccatgcggttaccagtgaagctataagtatgtagagctaacctcgtcttgcgcgcagatgcttgacctgtcgaagacgaaagacgagatgcgccggcgaacgaccgctttgcaccacatgcactaagaacgggcaccaatgcctcggttatcccgaggacaggagagatggcgaggcagcggcaaggacgggcgacgaggaaacgacgccaagggaggatgtcaaccaaggcgaggacgacgtcgcctctagaaaacccgctgcttcggggcttgcgaaccgtccgacgtcctctgggggcagcaatctgcaagctacgcatgctgctgcctctgctgcctctgcttcacggccgccgcggcgcaatatcaagcagactatcgaagtcggcgccgatgccaacccgggcgacgcagagccgcaacagtctcccgtactacatcaccaccaccagagccaccaccagaatcaccatcctcatcatcaagctcatctctcagtcacgtccgatgacttgcccagttcgcccaccctccgccgatcggcccccagccgtcgcatcccctatttccgctactttggctccacggccatcgtccccggcttcaagcaaatggtggtctctgttcgcgaccgtcgccgttcgacggcaggctcacattccggcgcctctcttcattcgacgcccagcggggcgatggccagtggctcggccattgacagcgacattgtccgcgaagacattccctcctacgaccccaacaactccgcccccgttcatcccttaatcattcagctagtcaatacgttttttgttcacgtcgggtgcaattacccctttctcaaacaagacaagtttctgcaacatgtaaaggagaaacgggtcgagccgatacttgtcgatgccgtctgcgccatcgcggcgcgcttctcggaccatcacatcctgacgggcggcaacgacaagatgccccggacagagagaggccaggtctttgcgcaacgggccaggcaggccaccgtcgacactttcccttgcccttctgtgggtgcggtccaggcttgcctgctgatggcatacgagggcttcggggcggcccaggatagcgcgctgtggatgtatctgggcttggccattcgcatggcggttgatctcggtctccaaaagtgcgtgggcgttcaatatcaaggcgaaaaggacccttggtacacccggcatcgaagtcgggccaacgacgatgatcaggacagcccagaggcgcacaaggcggatgccgtcgacgcccctagcccggaggaacagaaggaggtagagcaggagcgcatatataccttctggtccgtcttcatcctggaccggctcatctcctctggcactggacggccggtcacgatccgcgacggcgactacgagctcgcctttcccgaatccagcgtcgacctcgctaccggatggccgaacccatttcctgttctcctccagatcatccacctctacggtcaagtgtgcgatgtgctgaacaatctccacgacgcccaagaccttacccaggacaagtgggatcagctatccgagatggagcatcgactcacgagaatgtacaagcactgggacccgcggcttcagttcaacgtcaacaactttaagacgtacctcggcatgggccagggcaccaactttatcctcctccacttttggttccacgcgctcttcatcatattgcatcaaccgactcttcttacccccttttgcgaactgcggagcgagctccagctgctctcggacagccgtgagctgagcatgagcagcgcaaagaccatctgcgacattttgtcctttgccgacttgatagatccgacgagttttattggcaacccattcacgaatcagcccatttatatcgcggcatgcgcatttctcatggaatcgagcgccaacaatgcatctgagggctcgtccagggagggctcgcctcccactcaagcgagtcgctccaggcaacagacgaagcactttaacaagcagtctcggcattcgcttctcgcgtcggccgccaaccagaattaccagcgatgctacaactccctgcagcagatccaggcgtactggggcggagtaggctatatcctcaccgcgctggaccagaagtcaaagggcaagtgggactgcgagacgtataccgtggaggagtatgagagcaccaagctgccccctcctcggccgtcgattggtgagcagctgtcgcggttcgagaagcagtcgtcgcccaagattgccggctcaccgattgcttggagtctgtccggcacggccaattcgcccaactccagcctgacactcatgtatcaggctctcaacgccagcgcaggcggccacactggattccctccgcctgtgcagtccgtggcgagggctgccaatggttcgccggggagcatcgcgctggaccccattcgacacacgatgccggaagtgggaatgtttacgtcggcggttccgcagccaaacatgtctgccattcgaaactctcctcggcggccatatgctgccaattctatgaatgccgcgggggcgaactcgcggaatcagaatatcatgggcttcgaagacattccggaagagtcgccggatgcaaagggtctgatgtccaattactcaacctctggccagccctacgatggatataatgcatccccgaccagcggcaattcgggcatgggcaattctacagccgtgacgagtgcccccagtggaaacacgacgtcgaatgcgaatacccacaacaataacaacaacaacagcaccaccaccaccagcagcagcaacagcaacagcatgtatttcgcgcaaaacatggcatcatatcaagcctgggggccgatgacgggcaacatggacgccatcacgttcgacagccaggacattgacattgaggcgctggggctgcagcagccggacctgatgagcgggtggctcgagtatcttcccagtgatgtgctggggctgtttgacgagcatggcgagtcggggcagggcggccattga

SEQ ID NO: 14 - protein, 983 aa, Trichoderma reesei
MTTLLNNPPDSGPPPRQIRFVHNQGQPPSKRRRINAACLTCRRRKTRCAGERPLCTTCTKNGHQCLGYPEDRRDGEAAARTGDEETTPREDVNQGEDDVASRKPAASGLANRPTSSGGSNLQATHAAASAASASRPPRRNIKQTIENHHPHHQAHLSVTSDDLPSSPTLRRSAPSRRIPYFRYFGSTAIVPGFKQMVVSVRDRRRSTAGSHSGASLHSTPSGAMASGSAIDSDIVREDIPSYDPNNSAPVHPLIIQLVNTFFVHVGCNYPFLKQDKFLQHVKEKRVEPILVDAVCAIAARFSDHHILTGGNDKMPRTERGQVFAQRARQATVDTFPCPSVGAVQACLLMAYEGFGAAQDSALWMYLGLAIRMAVDLGLQKCVGVQYQGEKDPWYTRHRSRANDDDQDSPEAHKADAVDAPSPEEQKEVEQERIYTFWSVFILDRLISSGTGRPVTIRDGDYELAFPESSVDLATGWPNPFPVLLQIIHLYGQVCDVLNNLHDAQDLTQDKWDQLSEMEHRLTRMYKHWDPRLQFNVNNFKTYLGMGQGTNFILLHFWFHALFIILHQPTLLTPFCELRSELQLLSDSRELSMSSAKTICDILSFADLIDPTSFIGNPFTNQPIYIAACAFLMESSANNASEGSSREGSPPTQASRSRQQTKHFNKQSRHSLLASAANQNYQRCYNSLQQIQAYWGGVGYILTALDQKSKGKWDCETYTVEEYESTKLPPPRPSIGEQLSRFEKQSSPKIAGSPIAWSLSGTANSPNSSLTLMYQALNASAGGHTGFPPPVQSVARAANGSPGSIALDPIRHTMPEVGMFTSAVPQPNMSAIRNSPRRPYAANSMNAAGANSRNQNIMGFEDIPEESPDAKGLMSNYSTSGQPYDGYNASPTSGNSGMGNSTAVTSAPSGNTTNSMYFAQNMASYQAWGPMTGNMDAITFDSQDIDIEALGLQQPDLMSGWLEYLPSDVLGLFDEHGESGQGGH

SEQ ID NO: 15 - DNA, 1773 bp, Trichoderma reesei
atgtcaaccagacacatttttacgtcatgtgacggcctcgtcaacaaggccatccgaggcatcattacctacaacccttctctcagcctagacgaaagcaaccgggtcgtctatgacaccacatacgacaagtccaaagtcgtcatcataagcggaggcggctccggacatgagcctgcgtggacaggctatgtcggtcaaaacatgctcgcagcttcggttcaaggagacatctttgccagccccagcacaaagcaaatccttgcagcagtggacgctgttccgagtgacaagggcaccattctggtcatcacaaactacactggtgactgtctgcactttgggctggccaacgagaaagccaatgccaaaggccacaactgccggaccatcatctgcggcgacgatgtctctgtcggcaagaacgggagcatggttggtcgcagaggtttggctggacagatgggtgtcctcaaagtcatgggcggagctgctggtgctggaggctcgctggacgaagtttacaatcttggtgtcgcattctcgcagcagattgtgtctattgcggcaaccttggatcattgccatgttccaggacgtgctgaacatggcatgcttcaagaaggcgttgttgaactcggcaccggccctcataacgaacccggatacaagaaactatcccctgcgccatctgcgtctgatctcgtctcccagattctacaatactgtctgaatgaaaaggatccggaaagaggctacgttcacttcgcccctagtgatgaagtcatactacttctcagcaactacggcggcatatcgcacctggagatgggcgctctggttgacgaaattctcgagcagcttgcaagagactggaagattgagccggtgagggtatgcgccggcttcatcgagacgtcactcaatgctccagccttttctgtctccgtcatcaatgtgactgctgccgcaaagaattgcagttactctgtcgaagagatcaagtccttctttgatgccaggacgacgacgttttgggagtccatgactgggtcgcagacacggcggaggacgagacagcagcagattgttcagcccccggaggaagaggtcaaggcagttgatgagtcaaaagatctgactattgatcccacgctcttagagaagatgttgaggaacgcttgtgaagcgctcgtcaaggctgagccagatctcaccaagtgggataccgtcatgggtgatggagattgcggagagacgctcaggactggagccacatctttgctcacggcccttgattcgggattggcgaaatctgggtcagttgtgagagtactattggaactcgaagacatcgtggagagcaagatgggcggtactctgggcggcatattgggcatcttttttgtctccttgcgtgcagctgtcgagaagaatattggactggcccaaagcccggtcttgctctggggaacagctcttgcaacagctctggagagtctcaggaggtatacgcctgccaaggtcggagatcgtactgtcatggacacactcatcccgtttgctaccgtcatgtgtgagtcgggctttgataacggcgtcaaggcggcacaggatggagcggatgcgaccaagacgatgaagccgagactgggaagagcaacgtatgttggcgtgtcgagtgagaacaaggagttgcctcctgatcccggtgcttggggggccatggtggccattcgcggtttgcgacaaggtctggttgaagcgatctag

SEQ ID NO: 16 - protein, 590 aa, Trichoderma reesei
MSTRHIFTSCDGLVNKAIRGIITYNPSLSLDESNRVVYDTTYDKSKVVIISGGGSGHEPAWTGYVGQNMLAASVQGDIFASPSTKQILAAVDAVPSDKGTILVITNYTGDCLHFGLANEKANAKGHNCRTIICGDDVSVGKNGSMVGRRGLAGQMGVLKVMGGAAGAGGSLDEVYNLGVAFSQQIVSIAATLDHCHVPGRAEHGMLQEGVVELGTGPHNEPGYKKLSPAPSASDLVSQILQYCLNEKDPERGYVHFAPSDEVILLLSNYGGISHLEMGALVDEILEQLARDWKIEPVRVCAGFIETSLNAPAFSVSVINVTAAAKNCSYSVEEIKSFFDARTTTFWESMTGSQTRRRTRQQQIVQPPEEEVKAVDESKDLTIDPTLLEKMLRNACEALVKAEPDLTKWDTVMGDGDCGETLRTGATSLLTALDSGLAKSGSVVRVLLELEDIVESKMGGTLGGILGIFFVSLRAAVEKNIGLAQSPVLLWGTALATALESLRRYTPAKVGDRTVMDTLIPFATVMCESGFDNGVKAAQDGADATKTMKPRLGRATYVGVSSENKELPPDPGAWGAMVAIRGLRQGLVEAI

SEQ ID NO: 17 - DNA, 1326 bp, Trichoderma reesei
ttaggtgagggtgtaaccgccatcaacgcgaatatcggcaccggtcacatagcggctggcatcagacagcaggaaagccactgggcccatgagatcctgaggcagacccatcttgccctgaggaatgagggacacccatttcttcttcaggtcaggcttttcatccaggattttctcggtcctagttaaggatttgagttagccggccgaggtcacggctaccgttcaagaacagagaagagtgggttcaactcacaaagccgtcagcatgtatcccggcgagatacagttgactcggatgccagcatgcgcccactcaacggcgagcgaagccgcgagatggcggactgcggccttggaggcgttatagggcctagtccagttcaacccgttagctgtcttatgctctgctcatccatgtctcctttttttctttctttcttttttccgtcgtggaagggactcacgcttgaggctgggggacgttgacaatggcccccgacatgctgcctatcatgaccatgctaccagggctcttcctctccatgaggtgacgagcaaccgatgtagcgaagagatatgtgccgtcgacgttgacgccccagagcttgcgaactctatcaatggggtagttggtggcctcgaagttctcggtgaagccagccgaggtgaccaggttgtcaatcttgccatgttgctggatgatctcggcgatacacgcctcaacggaatcggcatctgagacgtcggcgtaatgcgccgtcactttgggaacgctagaccgggtgtcagccgtctgcctgcaaagccgtgttacgtgcagagcggagcggcagctcactcaccgttttgcgttggggttctccttgagaaaggcatccacgagcagtttcgtctgcttctcggcctcctcctctgtcgctgcgtcagctgtctggcctggggtacgagcgacccggaactggcacgcggaatctcactgttcatgtcgacgagggccaggtcggcgccagagaagaccattccctggccaatcaccagtcccagccctcttgcgccgccggtgacgacaccgacgtttccatcgagggagaagccggcaagcgtaggcttgacatactggccgccggtgccagagacgggctcgctgctcggaagctcatgctccggaggatactcgaactcgacctcggcgtcggttcgagagtggctgccgggcttatcctgccgcggcggcggcacactatggaacttcctcgcagcggccagcggcaggcgtctggcgggcgcggaggcaaaggttcggcgagccgcaagccgcagcat

SEQ ID NO: 18 - protein, 334 aa, Trichoderma reesei
MLRLAARRTFASAPARRLPLAAARKFHSVPPPRQDKPGSHSRTDAEVEFEYPPEHELPSSEPVSGTGGQYVKPTLAGFSLDGNVGVVTGGARGLGLVIGQGMVFSGADLALVDMNSEIPRASSGSLTADTRSSVPKVTAHYADVSDADSVEACIAEIIQQHGKIDNLVTSAGFTENFEATNYPIDRVRKLWGVNVDGTYLFATSVARHLMERKSPGSMVMIGSMSGAIVNVPQPQAPYNASKAAVRHLAASLAVEWAHAGIRVNCISPGYMLTALTEKILDEKPDLKKKWVSLIPQGKMGLPQDLMGPVAFLLSDASRYVTGADIRVDGGYTLT

SEQ ID NO: 19 - DNA, 640 bp, Trichoderma reesei
tcatgcctcaagatgcccaatctcttccaccttcttcgcactcgcactcgatggatcaaactcataccccagccactcagtagccaacctcctcgcaacttccagcccaacaaccctctcccccatacacaacacctgcgcattattgctctttacactgcgctcaacgctaaagctatcatgtgccgtaaccgctcgtatgcccttgaccttgttggcagaaatggcgacgcctagacctgtgccgcagatgagcagagcgcggtccgctttgccctcggcgacgaggcgggcggcggcggcggcgcgctggggatagggtgtcttgtcggagggctcgtcggatcctacgtcgatgacttggtctacgcgggcgtcgctttcaaagtcttttttgatggtgtttttgtagctgacgccggcgtcctgcggaagcgtgagtgagctcgtgtcagtgactgcccgttctgatgacctagattatgcaatcttgacgatgaagagaccgatagtcatgaagacttatgaagttgacacttgatctcgttgtgatatgagatgtgctggttctggcagccgaaacagaagcacttacatcgcagcccatggcgattctccatttcggtgccatcgtatatgt

SEQ ID NO: 20 - protein, 156 aa, Trichoderma reesei
TYTMAPKWRIAMGCDDAGVSYKNTIKKDFESDARVDQVIDVGSDEPSDKTPYPQRAAAAARLVAEGKADRALLICGTGLGVAISANKVKGIRAVTAHDSFSVERSVKSNNAQVLCMGERVVGLEVARRLATEWLGYEFDPSSASAKKVEEIGHLEA

SEQ ID NO: 21 - DNA, 726 bp, Trichoderma reesei
tcacgcttcagctacttcctgtatcgtcttgacaaactgctccggatcgtgtccgaaccgccccaggaacaatccgtccagtccgctcttcaacttctcgtagagccccggcccggcactccccccatacaaaaccctcgtcgtccccgccctcctcccaacggactccaaccctctgatcccagcaacaacatcgaggatgtgcttctctccagcaggttgactggcaccaatcgcccatacaggctcatacgccaaaatgacctctgcctcggcgggcacagcattcatgacagcatcaacctgcacccgacactcctcaaccgcgatatgcacgtcgccttgagtcttttctccaatgcacacaagcggtatcatgccattgcgacttacagcggcagccttattcgcaaccatggtgtcgtcctcgccaaagatgctcctgcgctctgcatgtccgacttccacgagcttgacgcctgcgctgcgcaacacggaggggctgacttcgccggtgaatgcgccttggtcttcccagtggcagtcttgagcgccggtccaaatggcaacggagctggacttaagctgggcgattgtggtggtcagggagacgaagtcggggatgatgaagatgtcaatgtgggagaggagctctatcgggacgtctgccagcttggataagaagctgtttgtgaagtctcttgtttgctggagagaaaagtacat

SEQ ID NO: 22 - protein, 241 aa, Trichoderma reesei
MYFSLQQTRDFTNSFLSKLADVPIELLSHIDIFIIPDFVSLTTTIAQLKSSSVAIWTGAQDCHWEDQGAFTGEVSPSVLRSAGVKLVEVGHAERRSIFGEDDTMVANKAAAVSRNGMIPLVCIGEKTQGDVHIAVEECRVQVDAVMNAVPAEAEVILAYEPVWAIGASQPAGEKHILDVVAGIRGLESVGRRAGTTRVLYGGSAGPGLYEKLKSGLDGLFLGRFGHDPEQFVKTIQEVAEA